European Patent Application EP 4 155 316 A1, published March 29, 2023. Title: HUMAN IL-15 MUTANT AND USES THEREOF. Applicant: JIANGSU SIMCERE PHARMACEUTICAL CO.,LTD. Application PCT/CN2021/094167. The sequence listing filed with the application follows.

SEQUENCE LISTING (100 sequences)

SEQ ID NO: 1 - protein, 114 aa, Artificial Sequence
NWVNVISDLKKIEDLIQSMHIDATLYTESDVHPSCKVTAMKCFLLELQVISLESGDASIHDTVENLIILANNSLSSNGNVTESGCKECEELEEKNIKEFLQSFVHIVQMFINTS

SEQ ID NO: 2 - DNA, 342 bp, Artificial Sequence
aactgggtgaatgtgatctctgacctgaagaagatcgaggatctgatccagtccatgcacatcgacgccaccctgtacacagagagcgatgtgcatccctcttgcaaggtgaccgctatgaagtgtttcctgctggagctgcaggtcatctctctggagtccggcgacgcctccatccacgataccgtggagaacctgatcatcctggctaacaattccctgtccagcaacggcaatgtgacagagagcggctgcaaggagtgtgaggagctggaggagaagaacatcaaggagttcctgcagagctttgtgcatatcgtgcagatgtttatcaatacatct

SEQ ID NO: 3 - protein, 114 aa, Artificial Sequence
NWVNVISELKKIEDLIQSMHIDATLYTESDVHPSCKVTAMKCFLLELQVISLESGDASIHDTVENLIILANNSLSSNGNVTESGCKECEELEEKNIKEFLQSFVHIVQMFINTS

SEQ ID NO: 4 - DNA, 342 bp, Artificial Sequence
aactgggtgaatgtgatctctgagctgaagaagatcgaggatctgatccagtccatgcacatcgacgccaccctgtacacagagagcgatgtgcatccctcttgcaaggtgaccgctatgaagtgtttcctgctggagctgcaggtcatctctctggagtccggcgacgcctccatccacgataccgtggagaacctgatcatcctggctaacaattccctgtccagcaacggcaatgtgacagagagcggctgcaaggagtgtgaggagctggaggagaagaacatcaaggagttcctgcagagctttgtgcatatcgtgcagatgtttatcaatacatct

SEQ ID NO: 5 - protein, 114 aa, Artificial Sequence
NWVNVISQLKKIEDLIQSMHIDATLYTESDVHPSCKVTAMKCFLLELQVISLESGDASIHDTVENLIILANNSLSSNGNVTESGCKECEELEEKNIKEFLQSFVHIVQMFINTS

SEQ ID NO: 6 - DNA, 342 bp, Artificial Sequence
aactgggtgaatgtgatctctcagctgaagaagatcgaggatctgatccagtccatgcacatcgacgccaccctgtacacagagagcgatgtgcatccctcttgcaaggtgaccgctatgaagtgtttcctgctggagctgcaggtcatctctctggagtccggcgacgcctccatccacgataccgtggagaacctgatcatcctggctaacaattccctgtccagcaacggcaatgtgacagagagcggctgcaaggagtgtgaggagctggaggagaagaacatcaaggagttcctgcagagctttgtgcatatcgtgcagatgtttatcaatacatct

SEQ ID NO: 7 - protein, 114 aa, Artificial Sequence
NWVNVISRLKKIEDLIQSMHIDATLYTESDVHPSCKVTAMKCFLLELQVISLESGDASIHDTVENLIILANNSLSSNGNVTESGCKECEELEEKNIKEFLQSFVHIVQMFINTS

SEQ ID NO: 8 - DNA, 342 bp, Artificial Sequence
aactgggtgaatgtgatctctaggctgaagaagatcgaggatctgatccagtccatgcacatcgacgccaccctgtacacagagagcgatgtgcatccctcttgcaaggtgaccgctatgaagtgtttcctgctggagctgcaggtcatctctctggagtccggcgacgcctccatccacgataccgtggagaacctgatcatcctggctaacaattccctgtccagcaacggcaatgtgacagagagcggctgcaaggagtgtgaggagctggaggagaagaacatcaaggagttcctgcagagctttgtgcatatcgtgcagatgtttatcaatacatct

SEQ ID NO: 9 - protein, 114 aa, Artificial Sequence
NWVNVISSLKKIEDLIQSMHIDATLYTESDVHPSCKVTAMKCFLLELQVISLESGDASIHDTVENLIILANNSLSSNGNVTESGCKECEELEEKNIKEFLQSFVHIVQMFINTS

SEQ ID NO: 10 - DNA, 342 bp, Artificial Sequence
aactgggtgaatgtgatctctagcctgaagaagatcgaggatctgatccagtccatgcacatcgacgccaccctgtacacagagagcgatgtgcatccctcttgcaaggtgaccgctatgaagtgtttcctgctggagctgcaggtcatctctctggagtccggcgacgcctccatccacgataccgtggagaacctgatcatcctggctaacaattccctgtccagcaacggcaatgtgacagagagcggctgcaaggagtgtgaggagctggaggagaagaacatcaaggagttcctgcagagctttgtgcatatcgtgcagatgtttatcaatacatct

SEQ ID NO: 11 - protein, 114 aa, Artificial Sequence
NWVNVISVLKKIEDLIQSMHIDATLYTESDVHPSCKVTAMKCFLLELQVISLESGDASIHDTVENLIILANNSLSSNGNVTESGCKECEELEEKNIKEFLQSFVHIVQMFINTS

SEQ ID NO: 12 - DNA, 342 bp, Artificial Sequence
aactgggtgaatgtgatctctgtgctgaagaagatcgaggatctgatccagtccatgcacatcgacgccaccctgtacacagagagcgatgtgcatccctcttgcaaggtgaccgctatgaagtgtttcctgctggagctgcaggtcatctctctggagtccggcgacgcctccatccacgataccgtggagaacctgatcatcctggctaacaattccctgtccagcaacggcaatgtgacagagagcggctgcaaggagtgtgaggagctggaggagaagaacatcaaggagttcctgcagagctttgtgcatatcgtgcagatgtttatcaatacatct

SEQ ID NO: 13 - protein, 114 aa, Artificial Sequence
NWLNVISDLKKIEDLIQSMHIDATLYTESDVHPSCKVTAMKCFLLELQVISLESGDASIHDTVENLIILANNSLSSNGNVTESGCKECEELEEKNIKEFLQSFVHIVQMFINTS

SEQ ID NO: 14 - DNA, 342 bp, Artificial Sequence
aactggctgaatgtgatctctgacctgaagaagatcgaggatctgatccagtccatgcacatcgacgccaccctgtacacagagagcgatgtgcatccctcttgcaaggtgaccgctatgaagtgtttcctgctggagctgcaggtcatctctctggagtccggcgacgcctccatccacgataccgtggagaacctgatcatcctggctaacaattccctgtccagcaacggcaatgtgacagagagcggctgcaaggagtgtgaggagctggaggagaagaacatcaaggagttcctgcagagctttgtgcatatcgtgcagatgtttatcaatacatct

SEQ ID NO: 15 - protein, 114 aa, Artificial Sequence
NWVNVDSDLKKIEDLIQSMHIDATLYTESDVHPSCKVTAMKCFLLELQVISLESGDASIHDTVENLIILANNSLSSNGNVTESGCKECEELEEKNIKEFLQSFVHIVQMFINTS

SEQ ID NO: 16 - DNA, 342 bp, Artificial Sequence
aactgggtgaatgtggactctgacctgaagaagatcgaggatctgatccagtccatgcacatcgacgccaccctgtacacagagagcgatgtgcatccctcttgcaaggtgaccgctatgaagtgtttcctgctggagctgcaggtcatctctctggagtccggcgacgcctccatccacgataccgtggagaacctgatcatcctggctaacaattccctgtccagcaacggcaatgtgacagagagcggctgcaaggagtgtgaggagctggaggagaagaacatcaaggagttcctgcagagctttgtgcatatcgtgcagatgtttatcaatacatct

SEQ ID NO: 17 - protein, 114 aa, Artificial Sequence
NWVNVISDLKKIEDLIQSMHIDATLYTESDVHPSCKVTAMKCFLLELQVISLESGDASIHDTVENLIILANNSLSSNGNVTESGCKECEELEEKNIKEFLQSFVKIVQMFINTS

SEQ ID NO: 18 - DNA, 342 bp, Artificial Sequence
aactgggtgaatgtgatctctgacctgaagaagatcgaggatctgatccagtccatgcacatcgacgccaccctgtacacagagagcgatgtgcatccctcttgcaaggtgaccgctatgaagtgtttcctgctggagctgcaggtcatctctctggagtccggcgacgcctccatccacgataccgtggagaacctgatcatcctggctaacaattccctgtccagcaacggcaatgtgacagagagcggctgcaaggagtgtgaggagctggaggagaagaacatcaaggagttcctgcagagctttgtgaagatcgtgcagatgtttatcaatacatct

SEQ ID NO: 19 - protein, 114 aa, Artificial Sequence
NWVNVISDLKKIEDLIQSMHIDATLYTESDVHPSCKVTAMKCFLLELQVISLESGDASIHDTVENLIILANNSLSSNGNVTESGCKECEELEEKNIKEFLQSFVNIVQMFINTS

SEQ ID NO: 20 - DNA, 342 bp, Artificial Sequence
aactgggtgaatgtgatctctgacctgaagaagatcgaggatctgatccagtccatgcacatcgacgccaccctgtacacagagagcgatgtgcatccctcttgcaaggtgaccgctatgaagtgtttcctgctggagctgcaggtcatctctctggagtccggcgacgcctccatccacgataccgtggagaacctgatcatcctggctaacaattccctgtccagcaacggcaatgtgacagagagcggctgcaaggagtgtgaggagctggaggagaagaacatcaaggagttcctgcagagctttgtgaacatcgtgcagatgtttatcaatacatct

SEQ ID NO: 21 - protein, 114 aa, Artificial Sequence
NWVNVISGLKKIEDLIQSMHIDATLYTESDVHPSCKVTAMKCFLLELQVISLESGDASIHDTVENLIILANNSLSSNGNVTESGCKECEELEEKNIKEFLQSFVHIVQMFINTS

SEQ ID NO: 22 - DNA, 342 bp, Artificial Sequence
aactgggtgaacgtgatctctggcctgaagaagatcgaggatctgatccagtctatgcacatcgatgccaccctgtacaccgagtctgatgtgcacccttcttgtaaggtgaccgccatgaagtgtttcctgctggagctgcaggtcatctctctggagtctggcgatgccagcatccacgataccgtggagaacctgatcatcctggccaacaactctctgtcttctaacggcaacgtgaccgagtctggctgtaaggagtgtgaggagctggaggagaagaacatcaaggagttcctgcagagcttcgtgcacatcgtgcagatgttcatcaacacctct

SEQ ID NO: 23 - protein, 114 aa, Artificial Sequence
NWVNVISILKKIEDLIQSMHIDATLYTESDVHPSCKVTAMKCFLLELQVISLESGDASIHDTVENLIILANNSLSSNGNVTESGCKECEELEEKNIKEFLQSFVHIVQMFINTS

SEQ ID NO: 24 - DNA, 342 bp, Artificial Sequence
aactgggtgaacgtgatctctatcctgaagaagatcgaggatctgatccagtctatgcacatcgatgccaccctgtacaccgagtctgatgtgcacccttcttgtaaggtgaccgccatgaagtgtttcctgctggagctgcaggtcatctctctggagtctggcgatgccagcatccacgataccgtggagaacctgatcatcctggccaacaactctctgtcttctaacggcaacgtgaccgagtctggctgtaaggagtgtgaggagctggaggagaagaacatcaaggagttcctgcagagcttcgtgcacatcgtgcagatgttcatcaacacctct

SEQ ID NO: 25 - protein, 114 aa, Artificial Sequence
NWVNVISLLKKIEDLIQSMHIDATLYTESDVHPSCKVTAMKCFLLELQVISLESGDASIHDTVENLIILANNSLSSNGNVTESGCKECEELEEKNIKEFLQSFVHIVQMFINTS

SEQ ID NO: 26 - DNA, 342 bp, Artificial Sequence
aactgggtgaacgtgatctctctgctgaagaagatcgaggatctgatccagtctatgcacatcgatgccaccctgtacaccgagtctgatgtgcacccttcttgtaaggtgaccgccatgaagtgtttcctgctggagctgcaggtcatctctctggagtctggcgatgccagcatccacgataccgtggagaacctgatcatcctggccaacaactctctgtcttctaacggcaacgtgaccgagtctggctgtaaggagtgtgaggagctggaggagaagaacatcaaggagttcctgcagagcttcgtgcacatcgtgcagatgttcatcaacacctct

SEQ ID NO: 27 - protein, 114 aa, Artificial Sequence
NWVNVPSDLKKIEDLIQSMHIDATLYTESDVHPSCKVTAMKCFLLELQVISLESGDASIHDTVENLIILANNSLSSNGNVTESGCKECEELEEKNIKEFLQSFVHIVQMFINTS

SEQ ID NO: 28 - DNA, 342 bp, Artificial Sequence
aactgggtgaacgtgccttctgatctgaagaagatcgaggatctgatccagtctatgcacatcgatgccaccctgtacaccgagtctgatgtgcacccttcttgtaaggtgaccgccatgaagtgtttcctgctggagctgcaggtcatctctctggagtctggcgatgccagcatccacgataccgtggagaacctgatcatcctggccaacaactctctgtcttctaacggcaacgtgaccgagtctggctgtaaggagtgtgaggagctggaggagaagaacatcaaggagttcctgcagagcttcgtgcacatcgtgcagatgttcatcaacacctct

SEQ ID NO: 29 - protein, 114 aa, Artificial Sequence
NWVNVISTLKKIEDLIQSMHIDATLYTESDVHPSCKVTAMKCFLLELQVISLESGDASIHDTVENLIILANNSLSSNGNVTESGCKECEELEEKNIKEFLQSFVHIVQMFINTS

SEQ ID NO: 30 - DNA, 342 bp, Artificial Sequence
aactgggtgaacgtgatctctaccctgaagaagatcgaggatctgatccagtctatgcacatcgatgccaccctgtacaccgagtctgatgtgcacccttcttgtaaggtgaccgccatgaagtgtttcctgctggagctgcaggtcatctctctggagtctggcgatgccagcatccacgataccgtggagaacctgatcatcctggccaacaactctctgtcttctaacggcaacgtgaccgagtctggctgtaaggagtgtgaggagctggaggagaagaacatcaaggagttcctgcagagcttcgtgcacatcgtgcagatgttcatcaacacctct

SEQ ID NO: 31 - protein, 429 aa, Artificial Sequence
NWVNVISDLKKIEDLIQSMHIDATLYTESDVHPSCKVTAMKCFLLELQVISCESGDASIHDTVENLIILANNSLSSNGNVTESGCKECEELEEKNIKEFLQSFVHIVQMFINTSITCPPPMSVEHADIWVKSYSLYSRERYICNSGFKRKAGTCSLTECVLNKATNVAHWTTPSLKCIRDPALVHQRGGGGSGGGGSEPKSSDKTHTCPPCPAPELLGGPSVFLFPPKPKDTLMISRTPEVTCVVVDVSHEDPEVKFNWYVDGVEVHNAKTKPREEQYNSTYRVVSVLTVLHQDWLNGKEYKCKVSNKALPAPIEKTISKAKGQPREPQVYTLPPSREEMTKNQVSLTCLVKGFYPSDIAVEWESNGQPENNYKTTPPVLDSDGSFFLYSKLTVDKSRWQQGNVFSCSVMHEALHNHYTQKSLSLSPGK

SEQ ID NO: 32 - DNA, 1287 bp, Artificial Sequence
aactgggtgaatgtgatctctgacctgaagaagatcgaggatctgatccagtccatgcacatcgacgccaccctgtacacagagagcgatgtgcatccctcttgcaaggtgaccgctatgaagtgtttcctgctggagctgcaggtcatctcttgcgagtccggcgacgcctccatccacgataccgtggagaacctgatcatcctggctaacaattccctgtccagcaacggcaatgtgacagagagcggctgcaaggagtgtgaggagctggaggagaagaacatcaaggagttcctgcagagctttgtgcatatcgtgcagatgtttatcaatacatctatcacctgcccccctccaatgtctgtggagcacgccgacatctgggtgaagtcctacagcctgtatagcagggagcggtacatctgtaactctggcttcaagaggaaggctggcacctgctccctgacagagtgcgtgctgaacaaggccacaaatgtggctcactggaccacacccagcctgaagtgcatcagagatcccgccctggtgcatcagagaggcggcggcggctctggcggcggcggctccgaacccaagtcctccgacaagacccacacctgtcccccttgtcctgcccctgaactgctgggcggaccttccgtgttcctgttccccccaaagcccaaggacaccctgatgatctcccggacccccgaagtgacctgcgtggtggtggatgtgtcccacgaggaccctgaagtgaagttcaattggtacgtggacggcgtggaagtgcacaacgccaagaccaagcctagagaggaacagtacaactccacctaccgggtggtgtccgtgctgacagtgctgcatcaggactggctgaacggcaaagagtacaagtgcaaggtgtccaacaaggccctgcctgcccccatcgaaaagaccatctccaaggccaagggccagccccgggaaccccaggtgtacacactgccccctagccgggaagagatgaccaagaaccaggtgtccctgacctgtctcgtgaaaggcttctacccctccgatatcgccgtggaatgggagtccaacggccagcctgagaacaactacaagaccaccccccctgtgctggactccgacggctcattcttcctgtacagcaagctgaccgtggacaagtcccggtggcagcagggcaacgtgttctcctgctccgtgatgcacgaggccctgcacaaccactacacccagaagtccctgtccctgagccccggcaag

SEQ ID NO: 33 - protein, 413 aa, Artificial Sequence
NWVNVISDLKKIEDLIQSMHIDATLYTESDVHPSCKVTAMKCFLLELQVISLESGDASIHDTVENLIILANDSLSSNGNVTESGCKECEELEEKNIKEFLQSFVHIVQMFINTSITCPPPMSVEHADIWVKSYSLYSRERYICNSGFKRKAGTSSLTECVLNKATNVAHWTTPSLKCIREFEPKSCDKTHTCPPCPAPELLGGPSVFLFPPKPKDTLMISRTPEVTCVVVDVSHEDPEVKFNWYVDGVEVHNAKTKPREEQYNSTYRVVSVLTVLHQDWLNGKEYKCKVSNKALPAPIEKTISKAKGQPREPQVYTLPPSREEMTKNQVSLTCLVKGFYPSDIAVEWESNGQPENNYKTTPPVLDSDGSFFLYSKLTVDKSRWQQGNVFSCSVMHEALHNHYTQKSLSLSPGK

SEQ ID NO: 34 - DNA, 1239 bp, Artificial Sequence
aactgggtgaatgtgatctctgacctgaagaagatcgaggatctgatccagtccatgcacatcgacgccaccctgtacacagagagcgatgtgcatccctcttgcaaggtgaccgctatgaagtgtttcctgctggagctgcaggtcatctctctggagtccggcgacgcctccatccacgataccgtggagaacctgatcatcctggctaatgactccctgtccagcaacggcaatgtgacagagagcggctgcaaggagtgtgaggagctggaggagaagaacatcaaggagttcctgcagagctttgtgcatatcgtgcagatgtttatcaatacatctatcacctgcccacctccaatgtccgtggagcacgctgacatctgggtgaagtcttactccctgtatagcagggagcggtacatctgcaactctggcttcaagagaaaggctggcacctccagcctgacagagtgcgtgctgaacaaggccacaaatgtggctcattggaccacacccagcctgaagtgtatccgcgagtttgaacccaagtcctgcgacaagacccacacctgtcccccttgtcctgcccctgaactgctgggcggaccttccgtgttcctgttccccccaaagcccaaggacaccctgatgatctcccggacccccgaagtgacctgcgtggtggtggatgtgtcccacgaggaccctgaagtgaagttcaattggtacgtggacggcgtggaagtgcacaacgccaagaccaagcctagagaggaacagtacaactccacctaccgggtggtgtccgtgctgacagtgctgcatcaggactggctgaacggcaaagagtacaagtgcaaggtgtccaacaaggccctgcctgcccccatcgaaaagaccatctccaaggccaagggccagccccgggaaccccaggtgtacacactgccccctagccgggaagagatgaccaagaaccaggtgtccctgacctgtctcgtgaaaggcttctacccctccgatatcgccgtggaatgggagtccaacggccagcctgagaacaactacaagaccaccccccctgtgctggactccgacggctcattcttcctgtacagcaagctgaccgtggacaagtcccggtggcagcagggcaacgtgttctcctgctccgtgatgcacgaggccctgcacaaccactacacccagaagtccctgtccctgagccccggcaag

SEQ ID NO: 35 - protein, 114 aa, Artificial Sequence
NWLNVISELKKIEDLIQSMHIDATLYTESDVHPSCKVTAMKCFLLELQVISLESGDASIHDTVENLIILANNSLSSNGNVTESGCKECEELEEKNIKEFLQSFVHIVQMFINTS

SEQ ID NO: 36 - DNA, 342 bp, Artificial Sequence
aactggctgaacgtcatcagtgagctgaagaagatcgaggacctgatccagtctatgcacatcgatgccaccctgtacaccgagtctgatgtgcacccttcttgtaaggtcaccgccatgaagtgtttcctgctggagctgcaggtcatctctctggagtctggcgatgcctctatccacgataccgtggagaacctgatcatcctggccaacaactctctgagctctaacggcaacgtaaccgagtctgggtgcaaggagtgtgaggagctggaggagaagaatatcaaggagtttctgcagtcttttgtgcacatcgtgcagatgtttatcaatacatct

SEQ ID NO: 37 - protein, 114 aa, Artificial Sequence
NWVNVDSELKKIEDLIQSMHIDATLYTESDVHPSCKVTAMKCFLLELQVISLESGDASIHDTVENLIILANNSLSSNGNVTESGCKECEELEEKNIKEFLQSFVHIVQMFINTS

SEQ ID NO: 38 - DNA, 342 bp, Artificial Sequence
aactgggtgaatgttgactctgagttgaagaaaattgaggacctaatccagtccatgcatatcgacgcaactctgtacactgagtctgacgtgcaccctagctgcaaagtgaccgccatgaagtgtttcctgctggagctgcaggtcatctctctggagtctggcgatgcctctatccacgatacagtggagaacctgatcatcctggccaacaactctctgagctctaacggaaacgtgaccgagtctggctgcaaggagtgtgaggagctggaggagaagaacatcaaggagttcctgcagtctttcgtgcatatcgtgcagatgttcatcaacacctct

SEQ ID NO: 39 - protein, 114 aa, Artificial Sequence
NWLNVDSDLKKIEDLIQSMHIDATLYTESDVHPSCKVTAMKCFLLELQVISLESGDASIHDTVENLIILANNSLSSNGNVTESGCKECEELEEKNIKEFLQSFVHIVQMFINTS

SEQ ID NO: 40 - DNA, 342 bp, Artificial Sequence
aactggctgaacgtggattctgatctgaagaagatcgaggatctgatccagtctatgcacatcgatgccacactgtacacagagtctgatgtgcacccttcttgtaaggtgaccgccatgaagtgttttctgctggagctgcaggtcatctctctggagtctggcgatgcctctatccacgataccgtggagaacctgatcatcctggccaacaactctctgagctctaacggcaacgtgaccgagtctggctgtaaggagtgtgaggagctggaggagaagaacatcaaggagtttctgcagtcttttgtgcacatcgtgcagatgtttatcaacacatct

SEQ ID NO: 41 - protein, 114 aa, Artificial Sequence
NWLNVDSDLKKIEDLIQSMHIDATLYTESDVHPSCKVTAMKCFLLELQVISLESGDASIHDTVENLIILANNSLSSNGNVTESGCKECEELEEKNIKEFLQSFVKIVQMFINTS

SEQ ID NO: 42 - DNA, 342 bp, Artificial Sequence
aactggctgaacgtggattctgatctgaagaagatcgaggatctgatccagtctatgcacatcgatgccaccctgtacaccgagtctgatgtgcacccttcttgtaaggtgaccgccatgaagtgtttcctgctggagctgcaggtcatctctctggagtctggcgatgcctctatccacgataccgtggagaacctgatcatcctggccaacaactctctgtctagcaacggcaacgtgaccgagtctggctgtaaggagtgtgaggagctggaggagaagaacatcaaggagttcctgcagtctttcgtgaagatcgtgcagatgttcatcaacacctct

SEQ ID NO: 43 - protein, 114 aa, Artificial Sequence
NWVNVDSDLKKIEDLIQSMHIDATLYTESDVHPSCKVTAMKCFLLELQVISLESGDASIHDTVENLIILANNSLSSNGNVTESGCKECEELEEKNIKEFLQSFVKIVQMFINTS

SEQ ID NO: 44 - DNA, 342 bp, Artificial Sequence
aactgggtgaacgtggattctgatctgaagaagatcgaggatctgatccagtctatgcacatcgatgccaccctgtacaccgagtctgatgtgcacccttcttgtaaggtgaccgccatgaagtgttttctgctggagctgcaggtcatctctctggagtctggcgatgcctctatccacgatacagtggagaacctgatcatcctggccaacaactctctgagctctaacggcaacgtgacagagtctggctgtaaggagtgtgaggagctggaggagaagaacatcaaggagtttctgcagtcttttgtgaagatcgtgcagatgtttatcaacacctct

SEQ ID NO: 45 - protein, 114 aa, Artificial Sequence
NWVNVISSLKKIEDLIQSMHIDATLYTESDVHPSCKVTAMKCFLLELQVISLESGDASIHDTVENLIILANNSLSSNGNVTESGCKECEELEEKNIKEFLQSFVKIVQMFINTS

SEQ ID NO: 46 - DNA, 342 bp, Artificial Sequence
aactgggtgaacgtgatctcttctctgaagaagatcgaggatctgatccagtctatgcacatcgatgccaccctgtacaccgagtctgatgtgcacccttcttgtaaggtgaccgccatgaagtgtttcctgctggagctgcaggtcatctctctggagtctggcgatgcctctatccacgataccgtggagaacctgatcatcctggccaacaactctctgagctctaacggcaacgtgaccgagtctggctgtaaggagtgtgaggagctggaggagaagaacatcaaggagttcctgcagtctttcgtgaagatcgtgcagatgttcatcaacacctct

SEQ ID NO: 47 - protein, 114 aa, Artificial Sequence
NWVNVISSLKKIEDLIQSMHIDATLYTESDVHPSCKVTAMKCFLLELQVISLESGDASIHDTVENLIILANNSLSSNGNVTESGCKECEELEEKNIKEFLQSFVNIVQMFINTS

SEQ ID NO: 48 - DNA, 342 bp, Artificial Sequence
aactgggtgaacgtgatctcttctctgaagaagatcgaggatctgatccagtctatgcacatcgatgccaccctgtacaccgagtctgatgtgcacccttcttgtaaggtgaccgccatgaagtgtttcctgctggagctgcaggtcatctctctggagtctggcgatgcctctatccacgataccgtggagaacctgatcatcctggccaacaactctctgagctctaacggcaacgtgaccgagtctggctgtaaggagtgtgaggagctggaggagaagaacatcaaggagttcctgcagtctttcgtgaacatcgtgcagatgttcatcaacacctct

SEQ ID NO: 49 - protein, 75 aa, Artificial Sequence
CPPPMSVEHADIWVKSYSLYSRERYICNSGFKRKAGTSSLTECVLNKATNVAHWTTPSLKCIRDPALVHQRPAPP

SEQ ID NO: 50 - DNA, 225 bp, Artificial Sequence
tgcccccctccaatgtctgtggagcacgccgacatctgggtgaagtcttactccctgtattccagggagcggtacatctgcaacagcggcttcaagaggaaggctggcacctccagcctgacagagtgcgtgctgaacaaggccaccaatgtggctcactggaccacaccttctctgaagtgtatcagagatccagccctggtgcatcagcgccccgctccccct

SEQ ID NO: 51 - protein, 63 aa, Artificial Sequence
CPPPMSVEHADIWVKSYSLYSRERYICNSGFKRKAGTSSLTECVLNKATNVAHWTTPSLKCIR

SEQ ID NO: 52 - DNA, 189 bp, Artificial Sequence
tgtcctcctcctatgtctgtggagcacgccgatatctgggtgaagtcttactctctgtactctagagagagatacatctgtaactctggcttcaagagaaaggccggcacctcttctctgaccgagtgtgtgctgaacaaggccaccaacgtggcccactggaccaccccttctctgaagtgtatcaga

SEQ ID NO: 53 - protein, 77 aa, Artificial Sequence
ITCPPPMSVEHADIWVKSYSLYSRERYICNSGFKRKAGTSSLTECVLNKATNVAHWTTPSLKCIRDPALVHQRPAPP

SEQ ID NO: 54 - DNA, 231 bp, Artificial Sequence
atcacatgtcctcctcctatgtctgtggagcacgctgatatttgggtgaagtcttactctctgtactctagagaaagatatatttgtaattctggctttaagagaaaggctggaacatcttctctgacagagtgtgtgctgaataaggctacaaacgtggctcattggacaacaccttctctgaagtgtattagagatcctgccctggtgcaccagagacctgctcctcct

SEQ ID NO: 55 - protein, 65 aa, Artificial Sequence
ITCPPPMSVEHADIWVKSYSLYSRERYICNSGFKRKAGTSSLTECVLNKATNVAHWTTPSLKCIR

SEQ ID NO: 56 - DNA, 195 bp, Artificial Sequence
atcacatgtcctcctcctatgtctgtggagcacgctgatatctgggtgaagtcttactctctgtactctagagagagatacatctgtaattctggctttaagagaaaggctggaacatcttctctgacagagtgtgtgctgaataaggctacaaatgtggctcactggacaacaccttctctgaagtgtatcaga

SEQ ID NO: 57 - protein, 448 aa, Artificial Sequence
EVQLVESGGGLVQPGGSLRLSCAASGFTFSDSWIHWVRQAPGKGLEWVAWISPYGGSTYYADSVKGRFTISADTSKNTAYLQMNSLRAEDTAVYYCARRHWPGGFDYWGQGTLVTVSSASTKGPSVFPLAPSSKSTSGGTAALGCLVKDYFPEPVTVSWNSGALTSGVHTFPAVLQSSGLYSLSSVVTVPSSSLGTQTYICNVNHKPSNTKVDKKVEPKSCDKTHTCPPCPAPELLGGPSVFLFPPKPKDTLMISRTPEVTCVVVDVSHEDPEVKFNWYVDGVEVHNAKTKPREEQYNSTYRVVSVLTVLHQDWLNGKEYKCKVSNKALPAPIEKTISKAKGQPREPQVYTLPPSREEMTKNQVSLTCLVKGFYPSDIAVEWESNGQPENNYKTTPPVLDSDGSFFLYSKLTVDKSRWQQGNVFSCSVMHEALHNHYTQKSLSLSPGK

SEQ ID NO: 58 - DNA, 1344 bp, Artificial Sequence
gaggtgcagctggtggagtccggaggaggactggtgcagccaggaggatccctgaggctgtcttgcgcagcaagcggcttcaccttttctgacagctggatccactgggtgcgccaggcaccaggcaagggactggagtgggtggcatggatcagcccttacggcggctccacctactatgccgactctgtgaagggccggttcacaatctccgccgatacctctaagaacacagcctatctgcagatgaatagcctgagggccgaggacacagccgtgtactattgtgcacggagacactggccaggaggatttgattactggggccagggcaccctggtgacagtgagctccgcttccaccaagggcccctccgtgtttcctctggccccttccagcaagtccacctctggcggaacagccgctctgggctgcctcgtgaaggactacttccccgagcccgtgacagtgtcttggaactctggcgccctgaccagcggagtgcacacctttccagctgtgctgcagtcctccggcctgtactccctgtcctccgtcgtgactgtgccctccagctctctgggcacccagacctacatctgcaacgtgaaccacaagccctccaacaccaaggtggacaagaaggtggaacccaagtcctgcgacaagacccacacctgtcccccttgtcctgcccctgaactgctgggcggaccttccgtgttcctgttccccccaaagcccaaggacaccctgatgatctcccggacccccgaagtgacctgcgtggtggtggatgtgtcccacgaggaccctgaagtgaagttcaattggtacgtggacggcgtggaagtgcacaacgccaagaccaagcctagagaggaacagtacgcctccacctaccgggtggtgtccgtgctgacagtgctgcatcaggactggctgaacggcaaagagtacaagtgcaaggtgtccaacaaggccctgcctgcccccatcgaaaagaccatctccaaggccaagggccagccccgggaaccccaggtgtacacactgccccctagccgggaagagatgaccaagaaccaggtgtccctgacctgtctcgtgaaaggcttctacccctccgatatcgccgtggaatgggagtccaacggccagcctgagaacaactacaagaccaccccccctgtgctggactccgacggctcattcttcctgtacagcaagctgaccgtggacaagtcccggtggcagcagggcaacgtgttctcctgctccgtgatgcacgaggccctgcacaaccactacacccagaagtccctgtccctgagccccggcaag

SEQ ID NO: 59 - protein, 214 aa, Artificial Sequence
DIQMTQSPSSLSASVGDRVTITCRASQDVSTAVAWYQQKPGKAPKLLIYSASFLYSGVPSRFSGSGSGTDFTLTISSLQPEDFATYYCQQYLYHPATFGQGTKVEIKRTVAAPSVFIFPPSDEQLKSGTASVVCLLNNFYPREAKVQWKVDNALQSGNSQESVTEQDSKDSTYSLSSTLTLSKADYEKHKVYACEVTHQGLSSPVTKSFNRGEC

SEQ ID NO: 60 - DNA, 642 bp, Artificial Sequence
gacatccagatgacccagtcccctagctccctgtccgcctctgtgggcgacagggtgaccatcacatgcagagcctctcaggatgtgagcacagcagtggcatggtaccagcagaagccaggcaaggcccctaagctgctgatctacagcgcctccttcctgtattccggcgtgccctctcggttttctggaagcggatccggaaccgacttcaccctgacaatctctagcctgcagccagaggattttgccacatactattgtcagcagtacctgtatcaccccgccaccttcggccagggcacaaaggtggagatcaagcggaccgtggccgctccctccgtgttcatcttcccaccttccgacgagcagctgaagtccggcaccgcttctgtcgtgtgcctgctgaacaacttctacccccgcgaggccaaggtgcagtggaaggtggacaatgccctgcagtccggcaactcccaggaatccgtgaccgagcaggactccaaggacagcacctactccctgtcctccaccctgaccctgtccaaggccgactacgagaagcacaaggtgtacgcctgcgaagtgacccaccagggcctgtctagccccgtgaccaagtctttcaaccggggcgagtgc

SEQ ID NO: 61 - protein, 448 aa, Artificial Sequence
QVQLQQSGPGLVKPSQTLSLTCAVSGDSITSGYWNWIRKFPSRGLEYMGYISYSGSTYYNPFLKSRISINRDTSKNQYYLQLNSVTPEDTAVYYCAKMGDWLAWFAYWGQGTLVTVSSASTKGPSVFPLAPSSKSTSGGTAALGCLVKDYFPEPVTVSWNSGALTSGVHTFPAVLQSSGLYSLSSVVTVPSSSLGTQTYICNVNHKPSNTKVDKKVEPKSCDKTHTCPPCPAPELLGGPSVFLFPPKPKDTLMISRTPEVTCVVVDVSHEDPEVKFNWYVDGVEVHNAKTKPREEQYNSTYRVVSVLTVLHQDWLNGKEYKCKVSNKALPAPIEKTISKAKGQPREPQVYTLPPSREEMTKNQVSLTCLVKGFYPSDIAVEWESNGQPENNYKTTPPVLDSDGSFFLYSKLTVDKSRWQQGNVFSCSVMHEALHNHYTQKSLSLSPGK

SEQ ID NO: 62 - DNA, 1344 bp, Artificial Sequence
caggtgcagctgcagcagtctggaccaggactggtgaagcctagccagaccctgtctctgacatgcgccgtgtctggcgactccatcaccagcggctattggaactggatcaggaagttcccatcccggggcctggagtacatgggctatatctcttactccggcagcacctactataacccctttctgaagtctagaatctccatcaaccgcgatacatccaagaatcagtactatctgcagctgaatagcgtgacccccgaggacacagccgtgtactattgtgctaagatgggcgattggctggcctggttcgcttactggggccagggcaccctggtgacagtgtccagcgcttccaccaagggcccctccgtgtttcctctggccccttccagcaagtccacctctggcggaacagccgctctgggctgcctcgtgaaggactacttccccgagcccgtgacagtgtcttggaactctggcgccctgaccagcggagtgcacacctttccagctgtgctgcagtcctccggcctgtactccctgtcctccgtcgtgactgtgccctccagctctctgggcacccagacctacatctgcaacgtgaaccacaagccctccaacaccaaggtggacaagaaggtggaacccaagtcctgcgacaagacccacacctgtcccccttgtcctgcccctgaactgctgggcggaccttccgtgttcctgttccccccaaagcccaaggacaccctgatgatctcccggacccccgaagtgacctgcgtggtggtggatgtgtcccacgaggaccctgaagtgaagttcaattggtacgtggacggcgtggaagtgcacaacgccaagaccaagcctagagaggaacagtacaactccacctaccgggtggtgtccgtgctgacagtgctgcatcaggactggctgaacggcaaagagtacaagtgcaaggtgtccaacaaggccctgcctgcccccatcgaaaagaccatctccaaggccaagggccagccccgggaaccccaggtgtacacactgccccctagccgggaagagatgaccaagaaccaggtgtccctgacctgtctcgtgaaaggcttctacccctccgatatcgccgtggaatgggagtccaacggccagcctgagaacaactacaagaccaccccccctgtgctggactccgacggctcattcttcctgtacagcaagctgaccgtggacaagtcccggtggcagcagggcaacgtgttctcctgctccgtgatgcacgaggccctgcacaaccactacacccagaagtccctgtccctgagccccggcaag

SEQ ID NO: 63 - protein, 220 aa, Artificial Sequence
EIVMTQSPPTLSLSPGERVTLSCKSSQSLLYSSNQKNSLAWYQQKPGQAPRLLIYWASTRESGIPARFSGSGSGTDFTLTISSLQPEDFAVYYCQQYYGYPYTFGQGTKLEIKRTVAAPSVFIFPPSDEQLKSGTASVVCLLNNFYPREAKVQWKVDNALQSGNSQESVTEQDSKDSTYSLSSTLTLSKADYEKHKVYACEVTHQGLSSPVTKSFNRGEC

SEQ ID NO: 64 - DNA, 660 bp, Artificial Sequence
gagatcgtgatgacccagtccccacctacactgtccctgagcccaggagagagagtgaccctgagctgcaagtccagccagtctctgctgtactcttccaaccagaagaattccctggcctggtatcagcagaagccaggacaggctccaaggctgctgatctactgggcttctaccagggagtccggaatccctgctcggttctctggatccggaagcggcacagactttaccctgacaatcagctctctgcagcctgaggatttcgccgtgtactattgtcagcagtactatggctacccatatacctttggccagggcacaaagctggagatcaagcggaccgtggccgctccctccgtgttcatcttcccaccttccgacgagcagctgaagtccggcaccgcttctgtcgtgtgcctgctgaacaacttctacccccgcgaggccaaggtgcagtggaaggtggacaatgccctgcagtccggcaactcccaggaatccgtgaccgagcaggactccaaggacagcacctactccctgtcctccaccctgaccctgtccaaggccgactacgagaagcacaaggtgtacgcctgcgaagtgacccaccagggcctgtctagccccgtgaccaagtctttcaaccggggcgagtgc

SEQ ID NO: 65 - protein, 20 aa, Artificial Sequence
SGGSGGGGSGGGSGGGGSLQ

SEQ ID NO: 66 - DNA, 60 bp, Artificial Sequence
agcggcggctctggcggcggcggcagcggcggcggctctggcggcggcggctctctgcag

SEQ ID NO: 67 - protein, 15 aa, Artificial Sequence
GGGGSGGGGSGGGGS

SEQ ID NO: 68 - DNA, 45 bp, Artificial Sequence
ggcggcggcggaagcggcggcggcggctctggcggcggcggctct

SEQ ID NO: 69 - protein, 2 aa, Artificial Sequence
EF

SEQ ID NO: 70 - DNA, 6 bp, Artificial Sequence
gagttc

SEQ ID NO: 71 - protein, 26 aa, Artificial Sequence
SGGGSGGGGSGGGGSGGGGSGGGSLQ

SEQ ID NO: 72 - DNA, 78 bp, Artificial Sequence
tctggaggcggcagcggcggcggcggctctggaggcggcggcagcggcggcggcggctctggcggcggatctctgcag

SEQ ID NO: 73 - protein, 232 aa, Artificial Sequence
EPKSSDKTHTCPPCPAPEAAGGPSVFLFPPKPKDTLMISRTPEVTCVVVDVSHEDPEVKFNWYVDGVEVHNAKTKPREEQYNSTYRVVSVLTVLHQDWLNGKEYKCKVSNKALPAPIEKTISKAKGQPREPQVYTLPPSREEMTKNQVSLTCLVKGFYPSDIAVEWESNGQPENNYKTTPPVLDSDGSFFLYSKLTVDKSRWQQGNVFSCSVMHEALHNHYTQKSLSLSPGK

SEQ ID NO: 74 - DNA, 696 bp, Artificial Sequence
gagcctaagtctagcgacaagacccacacctgtcccccttgtcctgcccctgaagccgccggcggaccttccgtgttcctgttccccccaaagcccaaggacaccctgatgatctcccggacccccgaagtgacctgcgtggtggtggatgtgtcccacgaggaccctgaagtgaagttcaattggtacgtggacggcgtggaagtgcacaacgccaagaccaagcctagagaggaacagtacaactccacctaccgggtggtgtccgtgctgacagtgctgcatcaggactggctgaacggcaaagagtacaagtgcaaggtgtccaacaaggccctgcctgcccccatcgaaaagaccatctccaaggccaagggccagccccgggaaccccaggtgtacacactgccccctagccgggaagagatgaccaagaaccaggtgtccctgacctgtctcgtgaaaggcttctacccctccgatatcgccgtggaatgggagtccaacggccagcctgagaacaactacaagaccaccccccctgtgctggactccgacggctcattcttcctgtacagcaagctgaccgtggacaagtcccggtggcagcagggcaacgtgttctcctgctccgtgatgcacgaggccctgcacaaccactacacccagaagtccctgtccctgagccccggcaag

SEQ ID NO: 75 - protein, 523 aa, Artificial Sequence
EVQLVESGGGLVQPGGSLRLSCAASGFTFSDSWIHWVRQAPGKGLEWVAWISPYGGSTYYADSVKGRFTISADTSKNTAYLQMNSLRAEDTAVYYCARRHWPGGFDYWGQGTLVTVSSASTKGPSVFPLAPSSKSTSGGTAALGCLVKDYFPEPVTVSWNSGALTSGVHTFPAVLQSSGLYSLSSVVTVPSSSLGTQTYICNVNHKPSNTKVDKKVEPKSCDKTHTCPPCPAPELLGGPSVFLFPPKPKDTLMISRTPEVTCVVVDVSHEDPEVKFNWYVDGVEVHNAKTKPREEQYNSTYRVVSVLTVLHQDWLNGKEYKCKVSNKALPAPIEKTISKAKGQPREPQVYTLPPSREEMTKNQVSLTCLVKGFYPSDIAVEWESNGQPENNYKTTPPVLDSDGSFFLYSKLTVDKSRWQQGNVFSCSVMHEALHNHYTQKSLSLSPGSCPPPMSVEHADIWVKSYSLYSRERYICNSGFKRKAGTSSLTECVLNKATNVAHWTTPSLKCIRDPALVHQRPAPP

SEQ ID NO: 76 - DNA, 1569 bp, Artificial Sequence
gaggtgcagctggtggagtccggaggaggactggtgcagccaggaggatccctgaggctgtcttgcgcagcaagcggcttcaccttttctgacagctggatccactgggtgcgccaggcaccaggcaagggactggagtgggtggcatggatcagcccttacggcggctccacctactatgccgactctgtgaagggccggttcacaatctccgccgatacctctaagaacacagcctatctgcagatgaatagcctgagggccgaggacacagccgtgtactattgtgcacggagacactggccaggaggatttgattactggggccagggcaccctggtgacagtgagctccgcttccaccaagggcccctccgtgtttcctctggccccttccagcaagtccacctctggcggaacagccgctctgggctgcctcgtgaaggactacttccccgagcccgtgacagtgtcttggaactctggcgccctgaccagcggagtgcacacctttccagctgtgctgcagtcctccggcctgtactccctgtcctccgtcgtgactgtgccctccagctctctgggcacccagacctacatctgcaacgtgaaccacaagccctccaacaccaaggtggacaagaaggtggaacccaagtcctgcgacaagacccacacctgtcccccttgtcctgcccctgaactgctgggcggaccttccgtgttcctgttccccccaaagcccaaggacaccctgatgatctcccggacccccgaagtgacctgcgtggtggtggatgtgtcccacgaggaccctgaagtgaagttcaattggtacgtggacggcgtggaagtgcacaacgccaagaccaagcctagagaggaacagtacaactccacctaccgggtggtgtccgtgctgacagtgctgcatcaggactggctgaacggcaaagagtacaagtgcaaggtgtccaacaaggccctgcctgcccccatcgaaaagaccatctccaaggccaagggccagccccgggaaccccaggtgtacacactgccccctagccgggaagagatgaccaagaaccaggtgtccctgacctgtctcgtgaaaggcttctacccctccgatatcgccgtggaatgggagtccaacggccagcctgagaacaactacaagaccaccccccctgtgctggactccgacggctcattcttcctgtacagcaagctgaccgtggacaagtcccggtggcagcagggcaacgtgttctcctgctccgtgatgcacgaggccctgcacaaccactacacccagaagtccctgtccctgagccccggcagctgcccccctccaatgtctgtggagcacgccgacatctgggtgaagtcttactccctgtattccagggagcggtacatctgcaacagcggcttcaagaggaaggctggcacctccagcctgacagagtgcgtgctgaacaaggccaccaatgtggctcactggaccacaccttctctgaagtgtatcagagatccagccctggtgcatcagcgccccgctccccct

SEQ ID NO: 77 - protein, 657 aa, Artificial Sequence
QVQLQQSGPGLVKPSQTLSLTCAVSGDSITSGYWNWIRKFPSRGLEYMGYISYSGSTYYNPFLKSRISINRDTSKNQYYLQLNSVTPEDTAVYYCAKMGDWLAWFAYWGQGTLVTVSSASTKGPSVFPLAPSSKSTSGGTAALGCLVKDYFPEPVTVSWNSGALTSGVHTFPAVLQSSGLYSLSSVVTVPSSSLGTQTYICNVNHKPSNTKVDKKVEPKSCDKTHTCPPCPAPELLGGPSVFLFPPKPKDTLMISRTPEVTCVVVDVSHEDPEVKFNWYVDGVEVHNAKTKPREEQYNSTYRVVSVLTVLHQDWLNGKEYKCKVSNKALPAPIEKTISKAKGQPREPQVYTLPPSREEMTKNQVSLTCLVKGFYPSDIAVEWESNGQPENNYKTTPPVLDSDGSFFLYSKLTVDKSRWQQGNVFSCSVMHEALHNHYTQKSLSLSPGSCPPPMSVEHADIWVKSYSLYSRERYICNSGFKRKAGTSSLTECVLNKATNVAHWTTPSLKCIRDPALVHQRPAPPSGGSGGGGSGGGSGGGGSLQNWVNVISDLKKIEDLIQSMHIDATLYTESDVHPSCKVTAMKCFLLELQVISLESGDASIHDTVENLIILANNSLSSNGNVTESGCKECEELEEKNIKEFLQSFVHIVQMFINTS

SEQ ID NO: 78 - DNA, 1971 bp, Artificial Sequence
caagtgcagctgcagcagtctggccctggcctggtgaagccttctcagaccctgtctctgacctgtgccgtgagcggcgattctatcacctctggctactggaactggatcagaaagtttccttctagaggcctggagtacatgggctacatctcttactctggctctacctactacaaccctttcctgaagtctagaatctctatcaacagagatacctctaagaaccagtactacctgcagctgaactctgtgacccctgaggataccgccgtgtactactgtgccaagatgggcgattggctggcctggttcgcctactggggccagggcaccctggtgaccgtgtcttctgctagcaccaagggcccatcggtcttccccctggcaccctcctccaagagcacctctgggggcacagcggccctgggctgcctggtcaaggactacttccccgaaccggtgacggtgtcgtggaactcaggcgccctgaccagcggcgtgcacaccttcccggctgtcctacagtcctcaggactctactccctcagcagcgtggtgaccgtgccctccagcagcttgggcacccagacctacatctgcaacgtgaatcacaagcccagcaacaccaaggtggacaagaaagttgagcccaaatcttgtgacaaaactcacacatgcccaccgtgcccagcacctgaactcctggggggaccgtcagtcttcctcttccccccaaaacccaaggacaccctcatgatctcccggacccccgaggtcacatgcgtggtggtggacgtgagccacgaagaccctgaggtcaagttcaactggtacgtggacggcgtggaggtgcataatgccaagacaaagccgcgggaggagcagtacaacagcacgtaccgtgtggtcagcgtcctcaccgtcctgcaccaggactggctgaatggcaaggagtacaagtgcaaggtctccaacaaagccctcccagcccccatcgagaaaaccatctccaaagccaaagggcagccccgagaaccacaggtgtacaccctgcccccatcccgggaggagatgaccaagaaccaggtcagcctgacctgcctggtcaaaggcttctatcccagcgacatcgccgtggagtgggagagcaatgggcagccggagaacaactacaagaccacgcctcccgtgctggactccgacggctccttcttcctctacagcaagctcaccgtggacaagagcaggtggcagcaggggaacgtcttctcatgctccgtgatgcatgaggctctgcacaaccactacacgcagaagagcctctccctgtctccgggtagctgcccccctccaatgtctgtggagcacgccgacatctgggtgaagtcttactccctgtattccagggagcggtacatctgcaacagcggcttcaagaggaaggctggcacctccagcctgacagagtgcgtgctgaacaaggccaccaatgtggctcactggaccacaccttctctgaagtgtatcagagatccagccctggtgcatcagcgccccgctccccctagcggcggctctggcggcggcggcagcggcggcggctctggcggcggcggctctctgcagaactgggtgaacgtgatctctgatctgaagaagatcgaggatctgatccagtctatgcacatcgatgccaccctgtacaccgagtctgatgtgcacccttcttgtaaggtgaccgccatgaagtgtttcctgctggagctgcaggtcatctctctggagtctggcgatgccagcatccacgataccgtggagaacctgatcatcctggccaacaactctctgtcttctaacggcaacgtgaccgagtctggctgtaaggagtgtgaggagctggaggagaagaacatcaaggagttcctgcagagcttcgtgcacatcgtgcagatgttcatcaacacctct

SEQ ID NO: 79 - protein, 657 aa, Artificial Sequence
QVQLQQSGPGLVKPSQTLSLTCAVSGDSITSGYWNWIRKFPSRGLEYMGYISYSGSTYYNPFLKSRISINRDTSKNQYYLQLNSVTPEDTAVYYCAKMGDWLAWFAYWGQGTLVTVSSASTKGPSVFPLAPSSKSTSGGTAALGCLVKDYFPEPVTVSWNSGALTSGVHTFPAVLQSSGLYSLSSVVTVPSSSLGTQTYICNVNHKPSNTKVDKKVEPKSCDKTHTCPPCPAPELLGGPSVFLFPPKPKDTLMISRTPEVTCVVVDVSHEDPEVKFNWYVDGVEVHNAKTKPREEQYNSTYRVVSVLTVLHQDWLNGKEYKCKVSNKALPAPIEKTISKAKGQPREPQVYTLPPSREEMTKNQVSLTCLVKGFYPSDIAVEWESNGQPENNYKTTPPVLDSDGSFFLYSKLTVDKSRWQQGNVFSCSVMHEALHNHYTQKSLSLSPGSCPPPMSVEHADIWVKSYSLYSRERYICNSGFKRKAGTSSLTECVLNKATNVAHWTTPSLKCIRDPALVHQRPAPPSGGSGGGGSGGGSGGGGSLQNWVNVISELKKIEDLIQSMHIDATLYTESDVHPSCKVTAMKCFLLELQVISLESGDASIHDTVENLIILANNSLSSNGNVTESGCKECEELEEKNIKEFLQSFVHIVQMFINTS

SEQ ID NO: 80 - DNA, 1971 bp, Artificial Sequence
caagtgcagctgcagcagtctggccctggcctggtgaagccttctcagaccctgtctctgacctgtgccgtgagcggcgattctatcacctctggctactggaactggatcagaaagtttccttctagaggcctggagtacatgggctacatctcttactctggctctacctactacaaccctttcctgaagtctagaatctctatcaacagagatacctctaagaaccagtactacctgcagctgaactctgtgacccctgaggataccgccgtgtactactgtgccaagatgggcgattggctggcctggttcgcctactggggccagggcaccctggtgaccgtgtcttctgctagcaccaagggcccatcggtcttccccctggcaccctcctccaagagcacctctgggggcacagcggccctgggctgcctggtcaaggactacttccccgaaccggtgacggtgtcgtggaactcaggcgccctgaccagcggcgtgcacaccttcccggctgtcctacagtcctcaggactctactccctcagcagcgtggtgaccgtgccctccagcagcttgggcacccagacctacatctgcaacgtgaatcacaagcccagcaacaccaaggtggacaagaaagttgagcccaaatcttgtgacaaaactcacacatgcccaccgtgcccagcacctgaactcctggggggaccgtcagtcttcctcttccccccaaaacccaaggacaccctcatgatctcccggacccccgaggtcacatgcgtggtggtggacgtgagccacgaagaccctgaggtcaagttcaactggtacgtggacggcgtggaggtgcataatgccaagacaaagccgcgggaggagcagtacaacagcacgtaccgtgtggtcagcgtcctcaccgtcctgcaccaggactggctgaatggcaaggagtacaagtgcaaggtctccaacaaagccctcccagcccccatcgagaaaaccatctccaaagccaaagggcagccccgagaaccacaggtgtacaccctgcccccatcccgggaggagatgaccaagaaccaggtcagcctgacctgcctggtcaaaggcttctatcccagcgacatcgccgtggagtgggagagcaatgggcagccggagaacaactacaagaccacgcctcccgtgctggactccgacggctccttcttcctctacagcaagctcaccgtggacaagagcaggtggcagcaggggaacgtcttctcatgctccgtgatgcatgaggctctgcacaaccactacacgcagaagagcctctccctgtctccgggtagctgcccccctccaatgtctgtggagcacgccgacatctgggtgaagtcttactccctgtattccagggagcggtacatctgcaacagcggcttcaagaggaaggctggcacctccagcctgacagagtgcgtgctgaacaaggccaccaatgtggctcactggaccacaccttctctgaagtgtatcagagatccagccctggtgcatcagcgccccgctccccctagcggcggctctggcggcggcggcagcggcggcggctctggcggcggcggctctctgcagaactgggtgaacgtgatctctgagctgaagaagatcgaggatctgatccagtctatgcacatcgatgccaccctgtacaccgagtctgatgtgcaccctagctgtaaggtgaccgccatgaagtgtttcctgctggagctgcaggtcatctctctggagtctggcgatgcctctatccacgataccgtggagaacctgatcatcctggccaacaactctctgtcctctaacggcaacgtgaccgagtctggctgtaaggagtgtgaggagctggaggagaagaacatcaaggagttcctgcagtctttcgtgcacatcgtgcagatgttcatcaacacctct

SEQ ID NO: 81 - protein, 657 aa, Artificial Sequence
QVQLQQSGPGLVKPSQTLSLTCAVSGDSITSGYWNWIRKFPSRGLEYMGYISYSGSTYYNPFLKSRISINRDTSKNQYYLQLNSVTPEDTAVYYCAKMGDWLAWFAYWGQGTLVTVSSASTKGPSVFPLAPSSKSTSGGTAALGCLVKDYFPEPVTVSWNSGALTSGVHTFPAVLQSSGLYSLSSVVTVPSSSLGTQTYICNVNHKPSNTKVDKKVEPKSCDKTHTCPPCPAPELLGGPSVFLFPPKPKDTLMISRTPEVTCVVVDVSHEDPEVKFNWYVDGVEVHNAKTKPREEQYNSTYRVVSVLTVLHQDWLNGKEYKCKVSNKALPAPIEKTISKAKGQPREPQVYTLPPSREEMTKNQVSLTCLVKGFYPSDIAVEWESNGQPENNYKTTPPVLDSDGSFFLYSKLTVDKSRWQQGNVFSCSVMHEALHNHYTQKSLSLSPGSCPPPMSVEHADIWVKSYSLYSRERYICNSGFKRKAGTSSLTECVLNKATNVAHWTTPSLKCIRDPALVHQRPAPPSGGSGGGGSGGGSGGGGSLQNWVNVISTLKKIEDLIQSMHIDATLYTESDVHPSCKVTAMKCFLLELQVISLESGDASIHDTVENLIILANNSLSSNGNVTESGCKECEELEEKNIKEFLQSFVHIVQMFINTS

SEQ ID NO: 82 - DNA, 1971 bp, Artificial Sequence
caagtgcagctgcagcagtctggccctggcctggtgaagccttctcagaccctgtctctgacctgtgccgtgagcggcgattctatcacctctggctactggaactggatcagaaagtttccttctagaggcctggagtacatgggctacatctcttactctggctctacctactacaaccctttcctgaagtctagaatctctatcaacagagatacctctaagaaccagtactacctgcagctgaactctgtgacccctgaggataccgccgtgtactactgtgccaagatgggcgattggctggcctggttcgcctactggggccagggcaccctggtgaccgtgtcttctgctagcaccaagggcccatcggtcttccccctggcaccctcctccaagagcacctctgggggcacagcggccctgggctgcctggtcaaggactacttccccgaaccggtgacggtgtcgtggaactcaggcgccctgaccagcggcgtgcacaccttcccggctgtcctacagtcctcaggactctactccctcagcagcgtggtgaccgtgccctccagcagcttgggcacccagacctacatctgcaacgtgaatcacaagcccagcaacaccaaggtggacaagaaagttgagcccaaatcttgtgacaaaactcacacatgcccaccgtgcccagcacctgaactcctggggggaccgtcagtcttcctcttccccccaaaacccaaggacaccctcatgatctcccggacccccgaggtcacatgcgtggtggtggacgtgagccacgaagaccctgaggtcaagttcaactggtacgtggacggcgtggaggtgcataatgccaagacaaagccgcgggaggagcagtacaacagcacgtaccgtgtggtcagcgtcctcaccgtcctgcaccaggactggctgaatggcaaggagtacaagtgcaaggtctccaacaaagccctcccagcccccatcgagaaaaccatctccaaagccaaagggcagccccgagaaccacaggtgtacaccctgcccccatcccgggaggagatgaccaagaaccaggtcagcctgacctgcctggtcaaaggcttctatcccagcgacatcgccgtggagtgggagagcaatgggcagccggagaacaactacaagaccacgcctcccgtgctggactccgacggctccttcttcctctacagcaagctcaccgtggacaagagcaggtggcagcaggggaacgtcttctcatgctccgtgatgcatgaggctctgcacaaccactacacgcagaagagcctctccctgtctccgggtagctgcccccctccaatgtctgtggagcacgccgacatctgggtgaagtcttactccctgtattccagggagcggtacatctgcaacagcggcttcaagaggaaggctggcacctccagcctgacagagtgcgtgctgaacaaggccaccaatgtggctcactggaccacaccttctctgaagtgtatcagagatccagccctggtgcatcagcgccccgctccccctagcggcggctctggcggcggcggcagcggcggcggctctggcggcggcggctctctgcagaactgggtgaacgtgatctctaccctgaagaagatcgaggatctgatccagtctatgcacatcgatgccaccctgtacaccgagtctgatgtgcacccttcttgtaaggtgaccgccatgaagtgtttcctgctggagctgcaggtcatctctctggagtctggcgatgccagcatccacgataccgtggagaacctgatcatcctggccaacaactctctgtcttctaacggcaacgtgaccgagtctggctgtaaggagtgtgaggagctggaggagaagaacatcaaggagttcctgcagagcttcgtgcacatcgtgcagatgttcatcaacacctct

SEQ ID NO: 83 - protein, 657 aa, Artificial Sequence
QVQLQQSGPGLVKPSQTLSLTCAVSGDSITSGYWNWIRKFPSRGLEYMGYISYSGSTYYNPFLKSRISINRDTSKNQYYLQLNSVTPEDTAVYYCAKMGDWLAWFAYWGQGTLVTVSSASTKGPSVFPLAPSSKSTSGGTAALGCLVKDYFPEPVTVSWNSGALTSGVHTFPAVLQSSGLYSLSSVVTVPSSSLGTQTYICNVNHKPSNTKVDKKVEPKSCDKTHTCPPCPAPELLGGPSVFLFPPKPKDTLMISRTPEVTCVVVDVSHEDPEVKFNWYVDGVEVHNAKTKPREEQYNSTYRVVSVLTVLHQDWLNGKEYKCKVSNKALPAPIEKTISKAKGQPREPQVYTLPPSREEMTKNQVSLTCLVKGFYPSDIAVEWESNGQPENNYKTTPPVLDSDGSFFLYSKLTVDKSRWQQGNVFSCSVMHEALHNHYTQKSLSLSPGSCPPPMSVEHADIWVKSYSLYSRERYICNSGFKRKAGTSSLTECVLNKATNVAHWTTPSLKCIRDPALVHQRPAPPSGGSGGGGSGGGSGGGGSLQNWVNVPSDLKKIEDLIQSMHIDATLYTESDVHPSCKVTAMKCFLLELQVISLESGDASIHDTVENLIILANNSLSSNGNVTESGCKECEELEEKNIKEFLQSFVHIVQMFINTS

SEQ ID NO: 84 - DNA, 1971 bp, Artificial Sequence
caagtgcagctgcagcagtctggccctggcctggtgaagccttctcagaccctgtctctgacctgtgccgtgagcggcgattctatcacctctggctactggaactggatcagaaagtttccttctagaggcctggagtacatgggctacatctcttactctggctctacctactacaaccctttcctgaagtctagaatctctatcaacagagatacctctaagaaccagtactacctgcagctgaactctgtgacccctgaggataccgccgtgtactactgtgccaagatgggcgattggctggcctggttcgcctactggggccagggcaccctggtgaccgtgtcttctgctagcaccaagggcccatcggtcttccccctggcaccctcctccaagagcacctctgggggcacagcggccctgggctgcctggtcaaggactacttccccgaaccggtgacggtgtcgtggaactcaggcgccctgaccagcggcgtgcacaccttcccggctgtcctacagtcctcaggactctactccctcagcagcgtggtgaccgtgccctccagcagcttgggcacccagacctacatctgcaacgtgaatcacaagcccagcaacaccaaggtggacaagaaagttgagcccaaatcttgtgacaaaactcacacatgcccaccgtgcccagcacctgaactcctggggggaccgtcagtcttcctcttccccccaaaacccaaggacaccctcatgatctcccggacccccgaggtcacatgcgtggtggtggacgtgagccacgaagaccctgaggtcaagttcaactggtacgtggacggcgtggaggtgcataatgccaagacaaagccgcgggaggagcagtacaacagcacgtaccgtgtggtcagcgtcctcaccgtcctgcaccaggactggctgaatggcaaggagtacaagtgcaaggtctccaacaaagccctcccagcccccatcgagaaaaccatctccaaagccaaagggcagccccgagaaccacaggtgtacaccctgcccccatcccgggaggagatgaccaagaaccaggtcagcctgacctgcctggtcaaaggcttctatcccagcgacatcgccgtggagtgggagagcaatgggcagccggagaacaactacaagaccacgcctcccgtgctggactccgacggctccttcttcctctacagcaagctcaccgtggacaagagcaggtggcagcaggggaacgtcttctcatgctccgtgatgcatgaggctctgcacaaccactacacgcagaagagcctctccctgtctccgggtagctgcccccctccaatgtctgtggagcacgccgacatctgggtgaagtcttactccctgtattccagggagcggtacatctgcaacagcggcttcaagaggaaggctggcacctccagcctgacagagtgcgtgctgaacaaggccaccaatgtggctcactggaccacaccttctctgaagtgtatcagagatccagccctggtgcatcagcgccccgctccccctagcggcggctctggcggcggcggcagcggcggcggctctggcggcggcggctctctgcagaactgggtgaacgtgccttctgatctgaagaagatcgaggatctgatccagtctatgcacatcgatgccaccctgtacaccgagtctgatgtgcacccttcttgtaaggtgaccgccatgaagtgtttcctgctggagctgcaggtcatctctctggagtctggcgatgccagcatccacgataccgtggagaacctgatcatcctggccaacaactctctgtcttctaacggcaacgtgaccgagtctggctgtaaggagtgtgaggagctggaggagaagaacatcaaggagttcctgcagagcttcgtgcacatcgtgcagatgttcatcaacacctct

SEQ ID NO: 85 - protein, 657 aa, Artificial Sequence
QVQLQQSGPGLVKPSQTLSLTCAVSGDSITSGYWNWIRKFPSRGLEYMGYISYSGSTYYNPFLKSRISINRDTSKNQYYLQLNSVTPEDTAVYYCAKMGDWLAWFAYWGQGTLVTVSSASTKGPSVFPLAPSSKSTSGGTAALGCLVKDYFPEPVTVSWNSGALTSGVHTFPAVLQSSGLYSLSSVVTVPSSSLGTQTYICNVNHKPSNTKVDKKVEPKSCDKTHTCPPCPAPELLGGPSVFLFPPKPKDTLMISRTPEVTCVVVDVSHEDPEVKFNWYVDGVEVHNAKTKPREEQYNSTYRVVSVLTVLHQDWLNGKEYKCKVSNKALPAPIEKTISKAKGQPREPQVYTLPPSREEMTKNQVSLTCLVKGFYPSDIAVEWESNGQPENNYKTTPPVLDSDGSFFLYSKLTVDKSRWQQGNVFSCSVMHEALHNHYTQKSLSLSPGSCPPPMSVEHADIWVKSYSLYSRERYICNSGFKRKAGTSSLTECVLNKATNVAHWTTPSLKCIRDPALVHQRPAPPSGGSGGGGSGGGSGGGGSLQNWLNVISELKKIEDLIQSMHIDATLYTESDVHPSCKVTAMKCFLLELQVISLESGDASIHDTVENLIILANNSLSSNGNVTESGCKECEELEEKNIKEFLQSFVHIVQMFINTS

SEQ ID NO: 86 - DNA, 1971 bp, Artificial Sequence
caagtgcagctgcagcagtctggccctggcctggtgaagccttctcagaccctgtctctgacctgtgccgtgagcggcgattctatcacctctggctactggaactggatcagaaagtttccttctagaggcctggagtacatgggctacatctcttactctggctctacctactacaaccctttcctgaagtctagaatctctatcaacagagatacctctaagaaccagtactacctgcagctgaactctgtgacccctgaggataccgccgtgtactactgtgccaagatgggcgattggctggcctggttcgcctactggggccagggcaccctggtgaccgtgtcttctgctagcaccaagggcccatcggtcttccccctggcaccctcctccaagagcacctctgggggcacagcggccctgggctgcctggtcaaggactacttccccgaaccggtgacggtgtcgtggaactcaggcgccctgaccagcggcgtgcacaccttcccggctgtcctacagtcctcaggactctactccctcagcagcgtggtgaccgtgccctccagcagcttgggcacccagacctacatctgcaacgtgaatcacaagcccagcaacaccaaggtggacaagaaagttgagcccaaatcttgtgacaaaactcacacatgcccaccgtgcccagcacctgaactcctggggggaccgtcagtcttcctcttccccccaaaacccaaggacaccctcatgatctcccggacccccgaggtcacatgcgtggtggtggacgtgagccacgaagaccctgaggtcaagttcaactggtacgtggacggcgtggaggtgcataatgccaagacaaagccgcgggaggagcagtacaacagcacgtaccgtgtggtcagcgtcctcaccgtcctgcaccaggactggctgaatggcaaggagtacaagtgcaaggtctccaacaaagccctcccagcccccatcgagaaaaccatctccaaagccaaagggcagccccgagaaccacaggtgtacaccctgcccccatcccgggaggagatgaccaagaaccaggtcagcctgacctgcctggtcaaaggcttctatcccagcgacatcgccgtggagtgggagagcaatgggcagccggagaacaactacaagaccacgcctcccgtgctggactccgacggctccttcttcctctacagcaagctcaccgtggacaagagcaggtggcagcaggggaacgtcttctcatgctccgtgatgcatgaggctctgcacaaccactacacgcagaagagcctctccctgtctccgggtagctgcccccctccaatgtctgtggagcacgccgacatctgggtgaagtcttactccctgtattccagggagcggtacatctgcaacagcggcttcaagaggaaggctggcacctccagcctgacagagtgcgtgctgaacaaggccaccaatgtggctcactggaccacaccttctctgaagtgtatcagagatccagccctggtgcatcagcgccccgctccccctagcggcggctctggcggcggcggcagcggcggcggctctggcggcggcggctctctgcagaactggctgaacgtcatcagtgagctgaagaagatcgaggacctgatccagtctatgcacatcgatgccaccctgtacaccgagtctgatgtgcacccttcttgtaaggtcaccgccatgaagtgtttcctgctggagctgcaggtcatctctctggagtctggcgatgcctctatccacgataccgtggagaacctgatcatcctggccaacaactctctgagctctaacggcaacgtaaccgagtctgggtgcaaggagtgtgaggagctggaggagaagaatatcaaggagtttctgcagtcttttgtgcacatcgtgcagatgtttatcaatacatct

SEQ ID NO: 87 - protein, 657 aa, Artificial Sequence
QVQLQQSGPGLVKPSQTLSLTCAVSGDSITSGYWNWIRKFPSRGLEYMGYISYSGSTYYNPFLKSRISINRDTSKNQYYLQLNSVTPEDTAVYYCAKMGDWLAWFAYWGQGTLVTVSSASTKGPSVFPLAPSSKSTSGGTAALGCLVKDYFPEPVTVSWNSGALTSGVHTFPAVLQSSGLYSLSSVVTVPSSSLGTQTYICNVNHKPSNTKVDKKVEPKSCDKTHTCPPCPAPELLGGPSVFLFPPKPKDTLMISRTPEVTCVVVDVSHEDPEVKFNWYVDGVEVHNAKTKPREEQYNSTYRVVSVLTVLHQDWLNGKEYKCKVSNKALPAPIEKTISKAKGQPREPQVYTLPPSREEMTKNQVSLTCLVKGFYPSDIAVEWESNGQPENNYKTTPPVLDSDGSFFLYSKLTVDKSRWQQGNVFSCSVMHEALHNHYTQKSLSLSPGSCPPPMSVEHADIWVKSYSLYSRERYICNSGFKRKAGTSSLTECVLNKATNVAHWTTPSLKCIRDPALVHQRPAPPSGGSGGGGSGGGSGGGGSLQNWLNVDSDLKKIEDLIQSMHIDATLYTESDVHPSCKVTAMKCFLLELQVISLESGDASIHDTVENLIILANNSLSSNGNVTESGCKECEELEEKNIKEFLQSFVHIVQMFINTS

SEQ ID NO: 88 - DNA, 1971 bp, Artificial Sequence
caagtgcagctgcagcagtctggccctggcctggtgaagccttctcagaccctgtctctgacctgtgccgtgagcggcgattctatcacctctggctactggaactggatcagaaagtttccttctagaggcctggagtacatgggctacatctcttactctggctctacctactacaaccctttcctgaagtctagaatctctatcaacagagatacctctaagaaccagtactacctgcagctgaactctgtgacccctgaggataccgccgtgtactactgtgccaagatgggcgattggctggcctggttcgcctactggggccagggcaccctggtgaccgtgtcttctgctagcaccaagggcccatcggtcttccccctggcaccctcctccaagagcacctctgggggcacagcggccctgggctgcctggtcaaggactacttccccgaaccggtgacggtgtcgtggaactcaggcgccctgaccagcggcgtgcacaccttcccggctgtcctacagtcctcaggactctactccctcagcagcgtggtgaccgtgccctccagcagcttgggcacccagacctacatctgcaacgtgaatcacaagcccagcaacaccaaggtggacaagaaagttgagcccaaatcttgtgacaaaactcacacatgcccaccgtgcccagcacctgaactcctggggggaccgtcagtcttcctcttccccccaaaacccaaggacaccctcatgatctcccggacccccgaggtcacatgcgtggtggtggacgtgagccacgaagaccctgaggtcaagttcaactggtacgtggacggcgtggaggtgcataatgccaagacaaagccgcgggaggagcagtacaacagcacgtaccgtgtggtcagcgtcctcaccgtcctgcaccaggactggctgaatggcaaggagtacaagtgcaaggtctccaacaaagccctcccagcccccatcgagaaaaccatctccaaagccaaagggcagccccgagaaccacaggtgtacaccctgcccccatcccgggaggagatgaccaagaaccaggtcagcctgacctgcctggtcaaaggcttctatcccagcgacatcgccgtggagtgggagagcaatgggcagccggagaacaactacaagaccacgcctcccgtgctggactccgacggctccttcttcctctacagcaagctcaccgtggacaagagcaggtggcagcaggggaacgtcttctcatgctccgtgatgcatgaggctctgcacaaccactacacgcagaagagcctctccctgtctccgggtagctgcccccctccaatgtctgtggagcacgccgacatctgggtgaagtcttactccctgtattccagggagcggtacatctgcaacagcggcttcaagaggaaggctggcacctccagcctgacagagtgcgtgctgaacaaggccaccaatgtggctcactggaccacaccttctctgaagtgtatcagagatccagccctggtgcatcagcgccccgctccccctagcggcggctctggcggcggcggcagcggcggcggctctggcggcggcggctctctgcagaactggctgaacgtggattctgatctgaagaagatcgaggatctgatccagtctatgcacatcgatgccacactgtacacagagtctgatgtgcacccttcttgtaaggtgaccgccatgaagtgttttctgctggagctgcaggtcatctctctggagtctggcgatgcctctatccacgataccgtggagaacctgatcatcctggccaacaactctctgagctctaacggcaacgtgaccgagtctggctgtaaggagtgtgaggagctggaggagaagaacatcaaggagtttctgcagtcttttgtgcacatcgtgcagatgtttatcaacacatct

SEQ ID NO: 89 - protein, 657 aa, Artificial Sequence
QVQLQQSGPGLVKPSQTLSLTCAVSGDSITSGYWNWIRKFPSRGLEYMGYISYSGSTYYNPFLKSRISINRDTSKNQYYLQLNSVTPEDTAVYYCAKMGDWLAWFAYWGQGTLVTVSSASTKGPSVFPLAPSSKSTSGGTAALGCLVKDYFPEPVTVSWNSGALTSGVHTFPAVLQSSGLYSLSSVVTVPSSSLGTQTYICNVNHKPSNTKVDKKVEPKSCDKTHTCPPCPAPELLGGPSVFLFPPKPKDTLMISRTPEVTCVVVDVSHEDPEVKFNWYVDGVEVHNAKTKPREEQYNSTYRVVSVLTVLHQDWLNGKEYKCKVSNKALPAPIEKTISKAKGQPREPQVYTLPPSREEMTKNQVSLTCLVKGFYPSDIAVEWESNGQPENNYKTTPPVLDSDGSFFLYSKLTVDKSRWQQGNVFSCSVMHEALHNHYTQKSLSLSPGSCPPPMSVEHADIWVKSYSLYSRERYICNSGFKRKAGTSSLTECVLNKATNVAHWTTPSLKCIRDPALVHQRPAPPSGGSGGGGSGGGSGGGGSLQNWLNVDSDLKKIEDLIQSMHIDATLYTESDVHPSCKVTAMKCFLLELQVISLESGDASIHDTVENLIILANNSLSSNGNVTESGCKECEELEEKNIKEFLQSFVKIVQMFINTS

SEQ ID NO: 90 - DNA, 1971 bp, Artificial Sequence
caagtgcagctgcagcagtctggccctggcctggtgaagccttctcagaccctgtctctgacctgtgccgtgagcggcgattctatcacctctggctactggaactggatcagaaagtttccttctagaggcctggagtacatgggctacatctcttactctggctctacctactacaaccctttcctgaagtctagaatctctatcaacagagatacctctaagaaccagtactacctgcagctgaactctgtgacccctgaggataccgccgtgtactactgtgccaagatgggcgattggctggcctggttcgcctactggggccagggcaccctggtgaccgtgtcttctgctagcaccaagggcccatcggtcttccccctggcaccctcctccaagagcacctctgggggcacagcggccctgggctgcctggtcaaggactacttccccgaaccggtgacggtgtcgtggaactcaggcgccctgaccagcggcgtgcacaccttcccggctgtcctacagtcctcaggactctactccctcagcagcgtggtgaccgtgccctccagcagcttgggcacccagacctacatctgcaacgtgaatcacaagcccagcaacaccaaggtggacaagaaagttgagcccaaatcttgtgacaaaactcacacatgcccaccgtgcccagcacctgaactcctggggggaccgtcagtcttcctcttccccccaaaacccaaggacaccctcatgatctcccggacccccgaggtcacatgcgtggtggtggacgtgagccacgaagaccctgaggtcaagttcaactggtacgtggacggcgtggaggtgcataatgccaagacaaagccgcgggaggagcagtacaacagcacgtaccgtgtggtcagcgtcctcaccgtcctgcaccaggactggctgaatggcaaggagtacaagtgcaaggtctccaacaaagccctcccagcccccatcgagaaaaccatctccaaagccaaagggcagccccgagaaccacaggtgtacaccctgcccccatcccgggaggagatgaccaagaaccaggtcagcctgacctgcctggtcaaaggcttctatcccagcgacatcgccgtggagtgggagagcaatgggcagccggagaacaactacaagaccacgcctcccgtgctggactccgacggctccttcttcctctacagcaagctcaccgtggacaagagcaggtggcagcaggggaacgtcttctcatgctccgtgatgcatgaggctctgcacaaccactacacgcagaagagcctctccctgtctccgggtagctgcccccctccaatgtctgtggagcacgccgacatctgggtgaagtcttactccctgtattccagggagcggtacatctgcaacagcggcttcaagaggaaggctggcacctccagcctgacagagtgcgtgctgaacaaggccaccaatgtggctcactggaccacaccttctctgaagtgtatcagagatccagccctggtgcatcagcgccccgctccccctagcggcggctctggcggcggcggcagcggcggcggctctggcggcggcggctctctgcagaactggctgaacgtggattctgatctgaagaagatcgaggatctgatccagtctatgcacatcgatgccaccctgtacaccgagtctgatgtgcacccttcttgtaaggtgaccgccatgaagtgtttcctgctggagctgcaggtcatctctctggagtctggcgatgcctctatccacgataccgtggagaacctgatcatcctggccaacaactctctgtctagcaacggcaacgtgaccgagtctggctgtaaggagtgtgaggagctggaggagaagaacatcaaggagttcctgcagtctttcgtgaagatcgtgcagatgttcatcaacacctct

SEQ ID NO: 91 - protein, 657 aa, Artificial Sequence
QVQLQQSGPGLVKPSQTLSLTCAVSGDSITSGYWNWIRKFPSRGLEYMGYISYSGSTYYNPFLKSRISINRDTSKNQYYLQLNSVTPEDTAVYYCAKMGDWLAWFAYWGQGTLVTVSSASTKGPSVFPLAPSSKSTSGGTAALGCLVKDYFPEPVTVSWNSGALTSGVHTFPAVLQSSGLYSLSSVVTVPSSSLGTQTYICNVNHKPSNTKVDKKVEPKSCDKTHTCPPCPAPELLGGPSVFLFPPKPKDTLMISRTPEVTCVVVDVSHEDPEVKFNWYVDGVEVHNAKTKPREEQYNSTYRVVSVLTVLHQDWLNGKEYKCKVSNKALPAPIEKTISKAKGQPREPQVYTLPPSREEMTKNQVSLTCLVKGFYPSDIAVEWESNGQPENNYKTTPPVLDSDGSFFLYSKLTVDKSRWQQGNVFSCSVMHEALHNHYTQKSLSLSPGSCPPPMSVEHADIWVKSYSLYSRERYICNSGFKRKAGTSSLTECVLNKATNVAHWTTPSLKCIRDPALVHQRPAPPSGGSGGGGSGGGSGGGGSLQNWVNVDSDLKKIEDLIQSMHIDATLYTESDVHPSCKVTAMKCFLLELQVISLESGDASIHDTVENLIILANNSLSSNGNVTESGCKECEELEEKNIKEFLQSFVKIVQMFINTS

SEQ ID NO: 92 - DNA, 1971 bp, Artificial Sequence
caagtgcagctgcagcagtctggccctggcctggtgaagccttctcagaccctgtctctgacctgtgccgtgagcggcgattctatcacctctggctactggaactggatcagaaagtttccttctagaggcctggagtacatgggctacatctcttactctggctctacctactacaaccctttcctgaagtctagaatctctatcaacagagatacctctaagaaccagtactacctgcagctgaactctgtgacccctgaggataccgccgtgtactactgtgccaagatgggcgattggctggcctggttcgcctactggggccagggcaccctggtgaccgtgtcttctgctagcaccaagggcccatcggtcttccccctggcaccctcctccaagagcacctctgggggcacagcggccctgggctgcctggtcaaggactacttccccgaaccggtgacggtgtcgtggaactcaggcgccctgaccagcggcgtgcacaccttcccggctgtcctacagtcctcaggactctactccctcagcagcgtggtgaccgtgccctccagcagcttgggcacccagacctacatctgcaacgtgaatcacaagcccagcaacaccaaggtggacaagaaagttgagcccaaatcttgtgacaaaactcacacatgcccaccgtgcccagcacctgaactcctggggggaccgtcagtcttcctcttccccccaaaacccaaggacaccctcatgatctcccggacccccgaggtcacatgcgtggtggtggacgtgagccacgaagaccctgaggtcaagttcaactggtacgtggacggcgtggaggtgcataatgccaagacaaagccgcgggaggagcagtacaacagcacgtaccgtgtggtcagcgtcctcaccgtcctgcaccaggactggctgaatggcaaggagtacaagtgcaaggtctccaacaaagccctcccagcccccatcgagaaaaccatctccaaagccaaagggcagccccgagaaccacaggtgtacaccctgcccccatcccgggaggagatgaccaagaaccaggtcagcctgacctgcctggtcaaaggcttctatcccagcgacatcgccgtggagtgggagagcaatgggcagccggagaacaactacaagaccacgcctcccgtgctggactccgacggctccttcttcctctacagcaagctcaccgtggacaagagcaggtggcagcaggggaacgtcttctcatgctccgtgatgcatgaggctctgcacaaccactacacgcagaagagcctctccctgtctccgggtagctgcccccctccaatgtctgtggagcacgccgacatctgggtgaagtcttactccctgtattccagggagcggtacatctgcaacagcggcttcaagaggaaggctggcacctccagcctgacagagtgcgtgctgaacaaggccaccaatgtggctcactggaccacaccttctctgaagtgtatcagagatccagccctggtgcatcagcgccccgctccccctagcggcggctctggcggcggcggcagcggcggcggctctggcggcggcggctctctgcagaactgggtgaacgtggattctgatctgaagaagatcgaggatctgatccagtctatgcacatcgatgccaccctgtacaccgagtctgatgtgcacccttcttgtaaggtgaccgccatgaagtgttttctgctggagctgcaggtcatctctctggagtctggcgatgcctctatccacgatacagtggagaacctgatcatcctggccaacaactctctgagctctaacggcaacgtgacagagtctggctgtaaggagtgtgaggagctggaggagaagaacatcaaggagtttctgcagtcttttgtgaagatcgtgcagatgtttatcaacacctct

SEQ ID NO: 93 - protein, 657 aa, Artificial Sequence
QVQLQQSGPGLVKPSQTLSLTCAVSGDSITSGYWNWIRKFPSRGLEYMGYISYSGSTYYNPFLKSRISINRDTSKNQYYLQLNSVTPEDTAVYYCAKMGDWLAWFAYWGQGTLVTVSSASTKGPSVFPLAPSSKSTSGGTAALGCLVKDYFPEPVTVSWNSGALTSGVHTFPAVLQSSGLYSLSSVVTVPSSSLGTQTYICNVNHKPSNTKVDKKVEPKSCDKTHTCPPCPAPELLGGPSVFLFPPKPKDTLMISRTPEVTCVVVDVSHEDPEVKFNWYVDGVEVHNAKTKPREEQYNSTYRVVSVLTVLHQDWLNGKEYKCKVSNKALPAPIEKTISKAKGQPREPQVYTLPPSREEMTKNQVSLTCLVKGFYPSDIAVEWESNGQPENNYKTTPPVLDSDGSFFLYSKLTVDKSRWQQGNVFSCSVMHEALHNHYTQKSLSLSPGSCPPPMSVEHADIWVKSYSLYSRERYICNSGFKRKAGTSSLTECVLNKATNVAHWTTPSLKCIRDPALVHQRPAPPSGGSGGGGSGGGSGGGGSLQNWVNVISSLKKIEDLIQSMHIDATLYTESDVHPSCKVTAMKCFLLELQVISLESGDASIHDTVENLIILANNSLSSNGNVTESGCKECEELEEKNIKEFLQSFVKIVQMFINTS

SEQ ID NO: 94 - DNA, 1971 bp, Artificial Sequence
caagtgcagctgcagcagtctggccctggcctggtgaagccttctcagaccctgtctctgacctgtgccgtgagcggcgattctatcacctctggctactggaactggatcagaaagtttccttctagaggcctggagtacatgggctacatctcttactctggctctacctactacaaccctttcctgaagtctagaatctctatcaacagagatacctctaagaaccagtactacctgcagctgaactctgtgacccctgaggataccgccgtgtactactgtgccaagatgggcgattggctggcctggttcgcctactggggccagggcaccctggtgaccgtgtcttctgctagcaccaagggcccatcggtcttccccctggcaccctcctccaagagcacctctgggggcacagcggccctgggctgcctggtcaaggactacttccccgaaccggtgacggtgtcgtggaactcaggcgccctgaccagcggcgtgcacaccttcccggctgtcctacagtcctcaggactctactccctcagcagcgtggtgaccgtgccctccagcagcttgggcacccagacctacatctgcaacgtgaatcacaagcccagcaacaccaaggtggacaagaaagttgagcccaaatcttgtgacaaaactcacacatgcccaccgtgcccagcacctgaactcctggggggaccgtcagtcttcctcttccccccaaaacccaaggacaccctcatgatctcccggacccccgaggtcacatgcgtggtggtggacgtgagccacgaagaccctgaggtcaagttcaactggtacgtggacggcgtggaggtgcataatgccaagacaaagccgcgggaggagcagtacaacagcacgtaccgtgtggtcagcgtcctcaccgtcctgcaccaggactggctgaatggcaaggagtacaagtgcaaggtctccaacaaagccctcccagcccccatcgagaaaaccatctccaaagccaaagggcagccccgagaaccacaggtgtacaccctgcccccatcccgggaggagatgaccaagaaccaggtcagcctgacctgcctggtcaaaggcttctatcccagcgacatcgccgtggagtgggagagcaatgggcagccggagaacaactacaagaccacgcctcccgtgctggactccgacggctccttcttcctctacagcaagctcaccgtggacaagagcaggtggcagcaggggaacgtcttctcatgctccgtgatgcatgaggctctgcacaaccactacacgcagaagagcctctccctgtctccgggtagctgcccccctccaatgtctgtggagcacgccgacatctgggtgaagtcttactccctgtattccagggagcggtacatctgcaacagcggcttcaagaggaaggctggcacctccagcctgacagagtgcgtgctgaacaaggccaccaatgtggctcactggaccacaccttctctgaagtgtatcagagatccagccctggtgcatcagcgccccgctccccctagcggcggctctggcggcggcggcagcggcggcggctctggcggcggcggctctctgcagaactgggtgaacgtgatctcttctctgaagaagatcgaggatctgatccagtctatgcacatcgatgccaccctgtacaccgagtctgatgtgcacccttcttgtaaggtgaccgccatgaagtgtttcctgctggagctgcaggtcatctctctggagtctggcgatgcctctatccacgataccgtggagaacctgatcatcctggccaacaactctctgagctctaacggcaacgtgaccgagtctggctgtaaggagtgtgaggagctggaggagaagaacatcaaggagttcctgcagtctttcgtgaagatcgtgcagatgttcatcaacacctct

SEQ ID NO: 95 - protein, 657 aa, Artificial Sequence
QVQLQQSGPGLVKPSQTLSLTCAVSGDSITSGYWNWIRKFPSRGLEYMGYISYSGSTYYNPFLKSRISINRDTSKNQYYLQLNSVTPEDTAVYYCAKMGDWLAWFAYWGQGTLVTVSSASTKGPSVFPLAPSSKSTSGGTAALGCLVKDYFPEPVTVSWNSGALTSGVHTFPAVLQSSGLYSLSSVVTVPSSSLGTQTYICNVNHKPSNTKVDKKVEPKSCDKTHTCPPCPAPELLGGPSVFLFPPKPKDTLMISRTPEVTCVVVDVSHEDPEVKFNWYVDGVEVHNAKTKPREEQYNSTYRVVSVLTVLHQDWLNGKEYKCKVSNKALPAPIEKTISKAKGQPREPQVYTLPPSREEMTKNQVSLTCLVKGFYPSDIAVEWESNGQPENNYKTTPPVLDSDGSFFLYSKLTVDKSRWQQGNVFSCSVMHEALHNHYTQKSLSLSPGSCPPPMSVEHADIWVKSYSLYSRERYICNSGFKRKAGTSSLTECVLNKATNVAHWTTPSLKCIRDPALVHQRPAPPSGGSGGGGSGGGSGGGGSLQNWVNVISSLKKIEDLIQSMHIDATLYTESDVHPSCKVTAMKCFLLELQVISLESGDASIHDTVENLIILANNSLSSNGNVTESGCKECEELEEKNIKEFLQSFVNIVQMFINTS

SEQ ID NO: 96 - DNA, 1971 bp, Artificial Sequence
caagtgcagctgcagcagtctggccctggcctggtgaagccttctcagaccctgtctctgacctgtgccgtgagcggcgattctatcacctctggctactggaactggatcagaaagtttccttctagaggcctggagtacatgggctacatctcttactctggctctacctactacaaccctttcctgaagtctagaatctctatcaacagagatacctctaagaaccagtactacctgcagctgaactctgtgacccctgaggataccgccgtgtactactgtgccaagatgggcgattggctggcctggttcgcctactggggccagggcaccctggtgaccgtgtcttctgctagcaccaagggcccatcggtcttccccctggcaccctcctccaagagcacctctgggggcacagcggccctgggctgcctggtcaaggactacttccccgaaccggtgacggtgtcgtggaactcaggcgccctgaccagcggcgtgcacaccttcccggctgtcctacagtcctcaggactctactccctcagcagcgtggtgaccgtgccctccagcagcttgggcacccagacctacatctgcaacgtgaatcacaagcccagcaacaccaaggtggacaagaaagttgagcccaaatcttgtgacaaaactcacacatgcccaccgtgcccagcacctgaactcctggggggaccgtcagtcttcctcttccccccaaaacccaaggacaccctcatgatctcccggacccccgaggtcacatgcgtggtggtggacgtgagccacgaagaccctgaggtcaagttcaactggtacgtggacggcgtggaggtgcataatgccaagacaaagccgcgggaggagcagtacaacagcacgtaccgtgtggtcagcgtcctcaccgtcctgcaccaggactggctgaatggcaaggagtacaagtgcaaggtctccaacaaagccctcccagcccccatcgagaaaaccatctccaaagccaaagggcagccccgagaaccacaggtgtacaccctgcccccatcccgggaggagatgaccaagaaccaggtcagcctgacctgcctggtcaaaggcttctatcccagcgacatcgccgtggagtgggagagcaatgggcagccggagaacaactacaagaccacgcctcccgtgctggactccgacggctccttcttcctctacagcaagctcaccgtggacaagagcaggtggcagcaggggaacgtcttctcatgctccgtgatgcatgaggctctgcacaaccactacacgcagaagagcctctccctgtctccgggtagctgcccccctccaatgtctgtggagcacgccgacatctgggtgaagtcttactccctgtattccagggagcggtacatctgcaacagcggcttcaagaggaaggctggcacctccagcctgacagagtgcgtgctgaacaaggccaccaatgtggctcactggaccacaccttctctgaagtgtatcagagatccagccctggtgcatcagcgccccgctccccctagcggcggctctggcggcggcggcagcggcggcggctctggcggcggcggctctctgcagaactgggtgaacgtgatctcttctctgaagaagatcgaggatctgatccagtctatgcacatcgatgccaccctgtacaccgagtctgatgtgcacccttcttgtaaggtgaccgccatgaagtgtttcctgctggagctgcaggtcatctctctggagtctggcgatgcctctatccacgataccgtggagaacctgatcatcctggccaacaactctctgagctctaacggcaacgtgaccgagtctggctgtaaggagtgtgaggagctggaggagaagaacatcaaggagttcctgcagtctttcgtgaacatcgtgcagatgttcatcaacacctct

SEQ ID NO: 97 - protein, 118 aa, Artificial Sequence
EVQLQESGPSLVKPSQTLSLTCSVTGDSITSGYWNWIRKFPGNKLEYMGYISYSGSTYYNPFLKSRISITRDTSKNQYYLQLNSVTTEDTATYYCAKMGDWLAWFAYWGQGTTVTVSS

SEQ ID NO: 98 - protein, 113 aa, Artificial Sequence
EIVMTQSPSSLAVSVGEKVTLSCKSSQSLLYSSNQKNSLAWYQQKPGQSPKLLIYWASTRESGVPDRFTGSGSGTDFTLTISSVKAEDLAVYYCQQYYGYPYTFGGGTKLEIK

SEQ ID NO: 99 - protein, 118 aa, Artificial Sequence
QVQLQQSGPGLVKPSQTLSLTCAVSGDSITSGYWNWIRKFPSRGLEYMGYISYSGSTYYNPFLKSRISINRDTSKNQYYLQLNSVTPEDTAVYYCAKMGDWLAWFAYWGQGTLVTVSS

SEQ ID NO: 100 - protein, 113 aa, Artificial Sequence
EIVMTQSPPTLSLSPGERVTLSCKSSQSLLYSSNQKNSLAWYQQKPGQAPRLLIYWASTRESGIPARFSGSGSGTDFTLTISSLQPEDFAVYYCQQYYGYPYTFGQGTKLEIK